European Patent Application EP 4 726 383 A1, published April 15, 2026. Title: Methods for detectig sesame. Applicant: NISSIN FOODS HOLDINGS. Application JP PNSH-00792. The sequence listing filed with the application follows.

SEQUENCE LISTING (3 sequences)

SEQ ID NO: 1 - protein, 9 aa, Sesamum indicum
ISGAQPSLR

SEQ ID NO: 2 - protein, 14 aa, Sesamum indicum
IQSEGGTTELWDER

SEQ ID NO: 3 - protein, 10 aa, Sesamum indicum
AFYLAGGVPR